European Patent Application EP 4 151 656 A1, published March 22, 2023. Title: HUMANIZED ANTI-IL-4R alpha SINGLE DOMAIN ANTIBODY AND APPLICATION THEREOF. Applicant: REGENECORE BIOTECH CO., LTD. The sequence listing filed with the application follows.

SEQUENCE LISTING (25 sequences)

SEQ ID NO: 1 - protein, 24 aa, artificial sequence
QVQLVESGGGSVQAGGSLRLSCAA

SEQ ID NO: 2 - protein, 24 aa, artificial sequence
QVQLVESGGGLVQPGGSLRLSCAA

SEQ ID NO: 3 - protein, 6 aa, artificial sequence
SGDFYC

SEQ ID NO: 4 - protein, 17 aa, artificial sequence
MAWFRQAPGKEREGVAT

SEQ ID NO: 5 - protein, 17 aa, artificial sequence
LGWFRQAPGQGLEAVAA

SEQ ID NO: 6 - protein, 17 aa, artificial sequence
LGWFRQAPGQEREAVAA

SEQ ID NO: 7 - protein, 17 aa, artificial sequence
MAWFRQAPGKEREAVAT

SEQ ID NO: 8 - protein, 16 aa, artificial sequence
MAWFRQAPGKEREAVA

SEQ ID NO: 9 - protein, 17 aa, artificial sequence
MAWFRQAPGKERERVAK

SEQ ID NO: 10 - protein, 17 aa, artificial sequence
MAWFRQAPGKERERVAT

SEQ ID NO: 11 - protein, 17 aa, artificial sequence
MAWFRQAPGKEREAVAA

SEQ ID NO: 12 - protein, 8 aa, artificial sequence
IRSGGRST

SEQ ID NO: 13 - protein, 38 aa, artificial sequence
YYADSVKGRFTISKDNAKDTLYLQMNSLKPEDTAMYYC

SEQ ID NO: 14 - protein, 38 aa, artificial sequence
YYADSVKGRFTISRDNSKNTLYLQMNSLRAEDTAVYYC

SEQ ID NO: 15 - protein, 38 aa, artificial sequence
YYADSVKGRFTISRDNSKNTLYLQMNSLKAEDTAVYYC

SEQ ID NO: 16 - protein, 38 aa, artificial sequence
YLADSVKGRFTISRDNSKNTLYLQMNSLKAEDTAVYYC

SEQ ID NO: 17 - protein, 38 aa, artificial sequence
YYADSVKGRFTISRDNSKNTVYLQMNSLKAEDTAVYYC

SEQ ID NO: 18 - protein, 12 aa, artificial sequence
AVGVDGNCRNYW

SEQ ID NO: 19 - protein, 12 aa, artificial sequence
AVGVDANCRNYW

SEQ ID NO: 20 - protein, 10 aa, artificial sequence
GQGTQVTVSS

SEQ ID NO: 21 - protein, 10 aa, artificial sequence
GQGTLVTVSS

SEQ ID NO: 22 - protein, 115 aa, artificial sequence
QVQLVESGGGSVQAGGSLRLSCAASGDFYCMAWFRQAPGKEREGVATIRSGGRSTYYADSVKGRFTISKDNAKDTLYLQMNSLKPEDTAMYYCAVGVDGNCRNYWGQGTQVTVSS

SEQ ID NO: 23 - DNA, 1434 bp, artificial sequence
caagtgcaacttgtggaatcaggaggaggatcagtgcaagcaggaggatcacttagactttcatgcgcagcatcaggagatttctattgtatggcatggtttagacaagcacctggaaaggagagggaaggagtggcaacaatcagatcaggaggaagatcaacatactacgcagattcagtgaaaggaagatttacaatctcaaaggacaatgcaaaggacaccctttaccttcaaatgaactcacttaaacctgaagatacagcaatgtactactgcgcagtgggagtggatggaaactgcagaaactactggggccaggggacacaagtgacagtgtcatcagagagcaagtacggccctccttgccccagctgccccgcccccgagtttctgggaggccccagcgtgtttctgtttcctcccaagcccaaagacacactgatgatcagcagaacccccgaggtgacatgcgtggtggtcgacgtgagccaagaagatcccgaggtgcagttcaactggtatgtggacggcgtggaggtgcacaacgccaagaccaagcctagggaggagcaattcaacagcacctacagagtggtgagcgtgctgaccgtgctgcaccaagactggctgaacggcaaggagtataagtgtaaggtgagcaacaagggcctccccagcagcatcgagaagaccatctccaaggccaagggccagcctagggagcctcaagtgtacacactgccccccagccaagaggagatgaccaaaaaccaagtgtctctgacatgcctcgtgaagggcttctatcccagcgacatcgccgtggagtgggagagcaatggccagcccgagaataactacaagaccaccccccccgtgctcgactccgatggcagcttctttctgtactctaggctgaccgtggacaagtctaggtggcaagagggaaacgtgttcagctgttccgtgatgcacgaggctctgcacaaccactacacccagaagagcctctctctgtctctgggaaaggagagcaagtacggccctccttgccccagctgcccccaagtgcagctggtggagagtgggggcggtagcgtacaagcgggcggcagcctgagactgagctgcgccgccagcggcaacaccttcagcttcagcacctactgcatgggctggttcagacagagccccggcaaggagagagagggcagcctggccaccatctacgacgccagcaccgcctacgccggcagcgtgaagggcagattcaccatcagcagagacaacagcaagaacatcctgtacctgcagatgaacaacctgagagccgaggacaccgccgtgtactactgcgccgccgccagatactgcatgttctggagccaccccagctactggggccagggcacccaggtgaccgtgagcagc

SEQ ID NO: 24 - protein, 478 aa, artificial sequence
QVQLVESGGGLVQPGGSLRLSCAASGDFYCMAWFRQAPGKEREAVAAIRSGGRSTYYADSVKGRFTISRDNSKNTLYLQMNSLKAEDTAVYYCAVGVDGNCRNYWGQGTLVTVSSESKYGPPCPSCPAPEFLGGPSVFLFPPKPKDTLMISRTPEVTCVVVDVSQEDPEVQFNWYVDGVEVHNAKTKPREEQFNSTYRVVSVLTVLHQDWLNGKEYKCKVSNKGLPSSIEKTISKAKGQPREPQVYTLPPSQEEMTKNQVSLTCLVKGFYPSDIAVEWESNGQPENNYKTTPPVLDSDGSFFLYSRLTVDKSRWQEGNVFSCSVMHEALHNHYTQKSLSLSLGKESKYGPPCPSCPQVQLVESGGGSVQAGGSLRLSCAASGNTFSFSTYCMGWFRQSPGKEREGSLATIYDASTAYAGSVKGRFTISRDNSKNILYLQMNNLRAEDTAVYYCAAARYCMFWSHPSYWGQGTQVTVSS

SEQ ID NO: 25 - protein, 122 aa, artificial sequence
QVQLVESGGGSVQAGGSLRLSCAASGNTFSFSTYCMGWFRQSPGKEREGSLATIYDGSTAYAGSVKGRFTISVDNAKNILYLQMNNLKPEDTAMYYCAAAKYCMFWSDPSYWGQGTQVTVSS